European Patent Application EP 4 643 875 A1, published November 5, 2025. Title: 이중나선 DNA가 결합된 금 나노 입자 운반체를 포함하는 백신 조성물. Applicant: 엔이에스바이오테크놀러지. The sequence listing filed with the application follows.

SEQUENCE LISTING (3 sequences)

SEQ ID NO: 1 - DNA, 720 bp, synthetic construct
  source 1..720: mol_type = other DNA
atgtttgtgttcctggtgctgctgccactggtgtccagccagtgtgtgagggtccaaccaacagagagcattgtgaggtttccaaacatcaccaacctgtgtccatttggagaggtgttcaatgccaccaggtttgcctctgtctatgcctggaacaggaagaggattagcaactgtgtggctgactactctgtgctctacaactctgcctccttcagcaccttcaagtgttatggagtgagcccaaccaaactgaatgacctgtgtttcaccaatgtctatgctgactcctttgtgattaggggagatgaggtgagacagattgcccctggacaaacaggcaagattgctgactacaactacaaactgcctgatgacttcacaggctgtgtgattgcctggaacagcaacaacctggacagcaaggtgggaggcaactacaactaccggtacagactgttcaggaagagcaacctgaaaccatttgagagggacatcagcacagagatttaccaggctggcagcaagccatgtaatggagtggagggcttcaactgttactttccactccaatcctatggcttccaaccaaccaatggagtgggctaccaaccatacagggtggtggtgctgtcctttgaactgctccatgcccctgccacagtgtgtggaccaaagaagagcaccaacctggtgaagaacaagtgtgtgaacttctga

SEQ ID NO: 2 - DNA, 1569 bp, synthetic construct
  source 1..1569: mol_type = other DNA
atggattggacttggatcttatttttagttgctgctgctactagagttcattctagcctgtggctgcccagcgaggccaccgtgtacctgccccccgtgcccgtgagcaaggtggtgagcaccgacgagtacgtggccaggaccaacatctactaccacgccggcaccagcaggctgctggccgtgggccacccctacttccccatcaagaagcccaacaacaacaagatcctggtgcccaaggtgagcggcctgcagtacagggtgttcaggatccacctgcccgaccccaacaagttcggcttccccgacaccagcttctacaaccccgacacccagaggctggtgtgggcctgcgtgggcgtggaggtgggcaggggccagcccctgggcgtgggcatcagcggccaccccctgctgaacaagctggacgacaccgagaacgccagcgcctacgccgccaacgccggcgtggacaacagggagtgcatcagcatggactacaagcagacccagctgtgcctgatcggctgcaagccccccatcggcgagcactggggcaagggcagcccctgcaccaacgtggccgtgaaccccggcgactgcccccccctggagctgatcaacaccgtgatccaggacggcgacatggtggacaccggcttcggcgccatggacttcaccaccctgcaggccaacaagagcgaggtgcccctggacatctgcaccagcatctgcaagtaccccgactacatcaagatggtgagcgagccctacggcgacagcctgttcttctacctgaggagggagcagatgttcgtgaggcacctgttcaacagggccggcgccgtgggcgagaacgtgcccgacgacctgtacatcaagggcagcggcagcaccgccaacctggccagcagcaactacttccccacccccagcggcagcatggtgaccagcgacgcccagatcttcaacaagccctactggctgcagagggcccagggccacaacaacggcatctgctggggcaaccagctgttcgtgaccgtggtggacaccaccaggagcaccaacatgagcctgtgcgccgccatcagcaccagcgagaccacctacaagaacaccaacttcaaggagtacctgaggcacggcgaggagtacgacctgcagttcatcttccagctgtgcaagatcaccctgaccgccgacgtgatgacctacatccacagcatgaacagcaccatcctggaggactggaacttcggcctgcagcccccccccggcggcaccctggaggacacctacaggttcgtgaccagccaggccatcgcctgccagaagcacaccccccccgcccccaaggaggaccccctgaagaagtacaccttctgggaggtgaacctgaaggagaagttcagcgccgacctggaccagttccccctgggcaggaagttcctgctgcaggccggcctgaaggccaagcccaagttcaccctgggcaagaggaaggccacccccaccaccagcagcaccagcaccaccgccaagaggaagaagaggaagctgtga

SEQ ID NO: 3 - DNA, 1576 bp, synthetic construct
  source 1..1576: mol_type = other DNA
atggattggacttggatcttatttttagttgctgctgctactagagttcattctgccctctggagaccatccgataacacagtgtacttgcccccacccagcgtcgcccgggtggtgaacacagacgactacgtcaccagaacctcaatcttctaccacgccgggtccagccggctgctgaccgtgggcaacccctacttccgcgtgcccgccggcggcggaaacaaacaagacatccccaaagtcagcgcctatcagtaccgggtgttccgcgtccaactgcccgatcccaacaagttcggcctgcccgacacctccatctacaaccccgagacccagaggctggtctgggcttgcgccggcgtcgagatcgggaggggccaacccctgggcgtggggttgtccggccaccccttctacaacaagctggacgataccgagtccagccacgcagcaaccagcaacgtctccgaagatgtgcgcgataacgtcagcgtggactacaaacaaacccaactgtgcatcctgggatgcgcacccgccatcggcgagcattgggccaaggggaccgcctgcaagagcaggcccctgagccaaggggactgtccacccctggagttgaagaataccgtgctcgaggacggcgacatggtggacaccggctacggcgctatggatttctccaccctccaggacaccaagtgcgaagtgcccctcgacatctgccaaagcatctgcaagtaccccgactacctccagatgagcgccgacccctacggcgacagcatgttcttctgtctcagaagggaacaattgttcgcccgccacttctggaaccgggccggcacaatgggagatacagtcccccagagcctgtacatcaaggggaccggaatgagggccagccccgggtcctgcgtctacagcccaagcccctccgggaacatcgtcacaagcgatagccaactcttcaacaagccctactggctccacaaagcccaaggccacaataacgggggtgtgttggcacaaccagctgttcgtgaccgtcgtggacacaaccaggtccacaaacctgaccatctgcgccagcacccaaagccccgtgcccggccagtacgacgccacaaagttcaaacaatactctcggcacgtggaagagtacgacctccaattcatcttccaactctgcaccatcaccctcaccgccgacgtgatgagctacatccactccatgaactcctccatcctggaagactggaatttcggcgtgccaccaccccctaccacctccctcgtcgacacctacagattcgtgcagagcgtggccatcacatgccagaaagacgccgcccccgccgagaacaaagacccatacgacaaactgaaattctggaacgtcgacctgaaagagaaattcagcctggatctggaccagtacccattgggcaggaagttcctcgtgcaagccggcctcaggagaaaaccaacaatcgggcccaggaagaggagcgcccccagcgcaaccaccagcagcaagcccgcaaaaagggtcagagtgagggcacgcaaatga